European Patent Application EP 4 265 726 A1, published October 25, 2023. Title: Deoxyribonucleoside and deoxyribonucleotide including new artificial base usable for screening of  DNA aptamer, and oligonucleotides containing thereof. Applicant: TAGCYX BIOTECHNOLOGIES INC. The sequence listing filed with the application follows.

SEQUENCE LISTING (20 sequences)

SEQ ID NO: 1 - DNA, 27 bp, Artificial Sequence
  synthetic DNA
ttctgtcaatcgatcgtatcagtccac

SEQ ID NO: 2 - DNA, 45 bp, Artificial Sequence
  synthetic DNA
  misc_feature (16)..(16): n is a linker consisting of alkylen group; -(CH2)12-, not a base, and not a nucleotide
tttttttttttttttnaagtagtcactaatccgttcgagtcatgc

SEQ ID NO: 3 - DNA, 102 bp, Artificial Sequence
  synthetic DNA
  misc_feature (50)..(50): n is synthetic base; Dsbn(7-(5-benzyl-2-thienyl)-3H-imidazo[4,5-b]pyridine)
  misc_feature (59)..(59): n is synthetic base; Dsbn(7-(5-benzyl-2-thienyl)-3H-imidazo[4,5-b]pyridine)
ttctgtcaatcgatcgtatcagtccacggtaaactgagtccgaaggggcntgcagtgancccgaatgggtccggcatgactcgaacggattagtgactactt

SEQ ID NO: 4 - DNA, 25 bp, Artificial Sequence
  synthetic DNA
ctccattgactcggcttaaactccc

SEQ ID NO: 5 - DNA, 41 bp, Artificial Sequence
  synthetic DNA
  misc_feature (16)..(16): n is a linker consisting of alkylen group; -(CH2)12-, not a base, and not a nucleotide
tttttttttttttttnagccaaggagcaccccaatatgacc

SEQ ID NO: 6 - DNA, 95 bp, Artificial Sequence
  synthetic DNA
  misc_feature (37)..(37): n is synthetic base; Dsbn(7-(5-benzyl-2-thienyl)-3H-imidazo[4,5-b]pyridine)
  misc_feature (47)..(47): n is synthetic base; Dsbn(7-(5-benzyl-2-thienyl)-3H-imidazo[4,5-b]pyridine)
ctccattgactcggcttaaactcccgtcagttatgantaggtacgcntgcggagttcgctaccccgccatggtcatattggggtgctccttggct

SEQ ID NO: 7 - DNA, 95 bp, Artificial Sequence; identical to SEQ ID NO: 6
  synthetic DNA
  misc_feature (37)..(37): n is synthetic base; Ds(7-(2-thienyl)imidazo[4,5-b]pyridine)
  misc_feature (47)..(47): n is synthetic base; Ds(7-(2-thienyl)imidazo[4,5-b]pyridine)

SEQ ID NO: 8 - DNA, 95 bp, Artificial Sequence
  synthetic DNA
ctccattgactcggcttaaactcccgtcagttatgaataggtacgcatgcggagttcgctaccccgccatggtcatattggggtgctccttggct

SEQ ID NO: 9 - DNA, 95 bp, Artificial Sequence
  synthetic DNA
  misc_feature (45)..(45): n is synthetic base; Dsbn(7-(5-benzyl-2-thienyl)-3H-imidazo[4,5-b]pyridine)
  misc_feature (57)..(57): n is synthetic base; Dsbn(7-(5-benzyl-2-thienyl)-3H-imidazo[4,5-b]pyridine)
ctccattgactcggcttaaactcccaggaggtggtgggggtgggnttagggttgggnttggaggggtgtcggtcatattggggtgctccttggct

SEQ ID NO: 10 - DNA, 95 bp, Artificial Sequence; identical to SEQ ID NO: 9
  synthetic DNA
  misc_feature (45)..(45): n is synthetic base; Ds(7-(2-thienyl)imidazo[4,5-b]pyridine)
  misc_feature (57)..(57): n is synthetic base; Ds(7-(2-thienyl)imidazo[4,5-b]pyridine)

SEQ ID NO: 11 - DNA, 95 bp, Artificial Sequence
  synthetic DNA
ctccattgactcggcttaaactcccaggaggtggtgggggtgggattagggttgggattggaggggtgtcggtcatattggggtgctccttggct

SEQ ID NO: 12 - DNA, 102 bp, Artificial Sequence; identical to SEQ ID NO: 3
  synthetic DNA
  misc_feature (50)..(50): n is synthetic base; Dscp(7-(5-(cyclopentylmethyl)thiophen-2-yl)-3H-imidazo[4,5-b]pyri dine)
  misc_feature (59)..(59): n is synthetic base; Dscp(7-(5-(cyclopentylmethyl)thiophen-2-yl)-3H-imidazo[4,5-b]pyri dine)

SEQ ID NO: 13 - DNA, 25 bp, Artificial Sequence
  synthetic DNA
gcgtgttgagctgtattagggtgtc

SEQ ID NO: 14 - DNA, 41 bp, Artificial Sequence
  synthetic DNA
  misc_feature (16)..(16): n is a linker consisting of alkylen group; -(CH2)12-, not a base, and not a nucleotide
tttttttttttttttnccgtctcatggatcaggattgtatc

SEQ ID NO: 15 - DNA, 95 bp, Artificial Sequence
  synthetic DNA
  misc_feature (45)..(45): n is synthetic base; Dscp(7-(5-(cyclopentylmethyl)thiophen-2-yl)-3H-imidazo[4,5-b]pyri dine)
  misc_feature (57)..(57): n is synthetic base; Dscp(7-(5-(cyclopentylmethyl)thiophen-2-yl)-3H-imidazo[4,5-b]pyri dine)
gcgtgttgagctgtattagggtgtcaggttttggtcaggcgttcnaacgtagaggantggacacttcggcgatacaatcctgatccatgagacgg

SEQ ID NO: 16 - DNA, 95 bp, Artificial Sequence; identical to SEQ ID NO: 15
  synthetic DNA
  misc_feature (45)..(45): n is synthetic base; Ds(7-(2-thienyl)imidazo[4,5-b]pyridine)
  misc_feature (57)..(57): n is synthetic base; Ds(7-(2-thienyl)imidazo[4,5-b]pyridine)

SEQ ID NO: 17 - DNA, 95 bp, Artificial Sequence
  synthetic DNA
gcgtgttgagctgtattagggtgtcaggttttggtcaggcgttcaaacgtagaggaatggacacttcggcgatacaatcctgatccatgagacgg

SEQ ID NO: 18 - DNA, 95 bp, Artificial Sequence
  Artificial
  misc_feature (45)..(45): n is synthetic base; Dscp(7-(5-(cyclopentylmethyl)thiophen-2-yl)-3H-imidazo[4,5-b]pyri dine)
  misc_feature (57)..(57): n is synthetic base; Dscp(7-(5-(cyclopentylmethyl)thiophen-2-yl)-3H-imidazo[4,5-b]pyri dine)
gcgtgttgagctgtattagggtgtcaggaaggattcgggggtggntttagggggggntcgttgtggaggcgatacaatcctgatccatgagacgg

SEQ ID NO: 19 - DNA, 95 bp, Artificial Sequence; identical to SEQ ID NO: 18
  synthetic DNA
  misc_feature (45)..(45): n is synthetic base; Ds(7-(2-thienyl)imidazo[4,5-b]pyridine)
  misc_feature (57)..(57): n is synthetic base; Ds(7-(2-thienyl)imidazo[4,5-b]pyridine)

SEQ ID NO: 20 - DNA, 95 bp, Artificial Sequence
  synthetic DNA
gcgtgttgagctgtattagggtgtcaggaaggattcgggggtggatttagggggggatcgttgtggaggcgatacaatcctgatccatgagacgg